European Patent Specification EP 3 546 573 B1, published January 15, 2025. Title: NUCLEASE-MEDIATED GENOME EDITING. Applicant: Wageningen Universiteit. The sequence listing filed with the application follows.

SEQUENCE LISTING (36 sequences)

SEQ ID NO: 1 - protein, 1304 aa, Artificial Sequence
  Cpf1 consensus sequence
  misc_feature (439)..(439): Xaa can be any naturally occurring amino acid
  misc_feature (504)..(504): Xaa can be any naturally occurring amino acid
  misc_feature (521)..(521): Xaa can be any naturally occurring amino acid
  misc_feature (539)..(539): Xaa can be any naturally occurring amino acid
  misc_feature (800)..(800): Xaa can be any naturally occurring amino acid
MSIYQEFVNKYSLSKTLRFELIPQGKTLENIKARGLILDDEKRAKDYKKAKQIIDKYHQFFIEEILSSVCISEDLLQNYSDVYFKLKKSDDDNLQKDFKSAKDTIKKQISEYIKDSEKFKNLFNQNLIDAKKGQESDLILWLKQSKDNGIELFKANSDITDIDEALEIIKSFKGWTTYFKGFHENRKNVYSSDDIPTSIIYRIVDDNLPKFLENKAKYESLKDKAPEAINYEQIKKDLAEELTFDIDYKTSEVNQRVFSLDEVFEIANFNNYLNQSGITKFNTIIGGKFVNGENTKRKGINEYINLYSQQINDKTLKKYKMSVLFKQILSDTESKSFVIDKLEDDSDVVTTMQSFYEQIAAFKTVEEKSIKETLSLLFDDLKAQKLDLSKIYFKNDKSLTDLSQQVFDDYSVIGTAVLEYITQQVAPKNLDNPSKKEQXLIAKKTEKAKYLSLETIKLALEEFNKHRDIDKQCRFEEILANFAAIPMIFDEIAQNKDNLAQISXKYQNQGKKDLLQASAEXDVKAIKDLLDQTNNLLHXLKIFHISQSEDKANILDKDEHFYLVFEECYFELANIVPLYNKIRNYITQKPYSDEKFKLNFENSTLANGWDKNKEPDNTAILFIKDDKYYLGVMNKKNNKIFDDKAIKENKGEGYKKIVYKLLPGANKMLPKVFFSAKSIKFYNPSEDILRIRNHSTHTKNGNPQKGYEKFEFNIEDCRKFIDFYKESISKHPEWKDFGFRFSDTQRYNSIDEFYREVENQGYKLTFENISESYIDSVVNQGKLYLFQIYNKDFSAYSKGXPNLHTLYWKALFDERNLQDVVYKLNGEAELFYRKQSIPKKITHPAKEAIANKNKDNPKKESVFEYDLIKDKRFTEDKFFFHCPITINFKSSGANKFNDEINLLLKEKANDVHILSIDRGERHLAYYTLVDGKGNIIKQDTFNIIGNDRMKTNYHDKLAAIEKDRDSARKDWKKINNIKEMKEGYLSQVVHEIAKLVIEYNAIVVFEDLNFGFKRGRFKVEKQVYQKLEKMLIEKLNYLVFKDNEFDKTGGVLRAYQLTAPFETFKKMGKQTGIIYYVPAGFTSKICPVTGFVNQLYPKYESVSKSQEFFSKFDKICYNLDKGYFEFSFDYKNFGDKAAKGKWTIASFGSRLINFRNSDKNHNWDTREVYPTKELEKLLKDYSIEYGHGECIKAAICGESDKKFFAKLTSVLNTILQMRNSKTGTELDYLISPVADVNGNFFDSRQAPKNMPQDADANGAYHIGLKGLMLLDRIKNNQEGKKLNLVIKNEEYFEFVQNRNNSSKI

SEQ ID NO: 2 - protein, 5 aa, Artificial Sequence
  Residues 786 - 791 of SEQ ID NO:1
FQIYN

SEQ ID NO: 3 - protein, 6 aa, Artificial Sequence
  Residues 786 - 791 of SEQ ID NO:1
FQIYNK

SEQ ID NO: 4 - protein, 7 aa, Artificial Sequence
  Residues 786 - 792 of SEQ ID NO:1
FQIYNKD

SEQ ID NO: 5 - protein, 14 aa, Artificial Sequence
  Residues 781 - 794 of SEQ ID NO:1
  misc_feature (1)..(1): Xaa can be Gly or Lys
  misc_feature (2)..(2): Xaa can be Lys, Ser or Asp
  misc_feature (3)..(3): Xaa can be Leu or Ile
  misc_feature (4)..(4): Xaa can be Tyr or Phe
  misc_feature (5)..(5): Xaa can be Leu or Met
  misc_feature (13)..(13): Xaa can be Phe or Tyr
  misc_feature (14)..(14): Xaa can be Ser, Ala or Val
XXXXXFQIYNKDXX

SEQ ID NO: 6 - protein, 14 aa, Artificial Sequence
  Residues 781 - 794 of SEQ ID NO:1
GKLYLFQIYNKDFS

SEQ ID NO: 7 - protein, 7 aa, Artificial Sequence
  RuvC domain of catalytically inactive Cpf1
  misc_feature (1)..(1): Xaa can be Gly or Ser
XIDRGER

SEQ ID NO: 8 - protein, 6 aa, Artificial Sequence
  RuvC domain of catalytically inactive Cpf1
DANGAY

SEQ ID NO: 9 - protein, 4 aa, Artificial Sequence
  RuvC domain of catalytically inactive Cpf1
  misc_feature (2)..(2): Xaa can be Asp, Asn or Glu
EXLN

SEQ ID NO: 10 - protein, 4 aa, Artificial Sequence
  RuvC domain of catalytically inactive Cpf1
EDLN

SEQ ID NO: 11 - protein, 7 aa, Artificial Sequence
  RuvC domain
SIDRGER

SEQ ID NO: 12 - protein, 7 aa, Artificial Sequence
  RuvC domain
GIDRGER

SEQ ID NO: 13 - protein, 4 aa, Artificial Sequence
  RuvC domain
ENLN

SEQ ID NO: 14 - protein, 4 aa, Artificial Sequence
  RuvC domain
EELN

SEQ ID NO: 15 - protein, 19 aa, Artificial Sequence
  Arginine-rich motif
  misc_feature (1)..(1): Xaa can be Asp or Asn
  misc_feature (3)..(3): Xaa can be Arg, Gln or His
  misc_feature (4)..(4): Xaa can be Lys, Glu, Ser or Asp
  misc_feature (5)..(5): Xaa can be Ala, Lys or Leu
  misc_feature (7)..(7): Xaa can be Asp, Asn or Ala
  misc_feature (8)..(8): Xaa can be Val, Asn, Gln, Lys, or Ala
  misc_feature (9)..(9): Xaa can be Arg, Lys or Ile
  misc_feature (11)..(11): Xaa can be Tyr, Lys or Ile
  misc_feature (12)..(12): Xaa can be Asp or Glu
  misc_feature (13)..(13): Xaa can be Asn, Arg or Met
  misc_feature (14)..(14): Xaa can be Lys, Val, Phe or Asp
  misc_feature (15)..(15): Xaa can be Glu, Ala, Asp or Ser
  misc_feature (18)..(18): Xaa can be Arg, Gln or Lys
  misc_feature (19)..(19): Xaa can be Asn, Ala, Ser or Asp
XYXXXLXXXEXXXXXARXX

SEQ ID NO: 16 - protein, 19 aa, Artificial Sequence
  Arginine-rich motif
DYRKALDVREYDNKEARRN

SEQ ID NO: 17 - protein, 19 aa, Artificial Sequence
  Arginine-rich motif
DYQKKLDNREKERVAARQA

SEQ ID NO: 18 - protein, 19 aa, Artificial Sequence
  Arginine-rich motif
DYREKLNQREIEMKDARQS

SEQ ID NO: 19 - protein, 19 aa, Artificial Sequence
  Arginine-rich motif
DYHSLLDKKEKERFEARQN

SEQ ID NO: 20 - protein, 19 aa, Artificial Sequence
  Arginine-rich motif
NYHDKLAAIEKDRDSARKD

SEQ ID NO: 21 - DNA, 29 bp, Francisella novicida
agattaaaaggtaattctatcttgttgag

SEQ ID NO: 22 - DNA, 45 bp, Francisella novicida
ataatttaagattaaaaggtaattctattttgttgagatctgagc

SEQ ID NO: 23 - DNA, 26 bp, Francisella novicida
tagcgatttatgaaggtcattttttt

SEQ ID NO: 24 - DNA, 42 bp, Francisella novicida
ctaaattatagcgatttatgaaggtcatttttttaaaaagtt

SEQ ID NO: 25 - DNA, 29 bp, Francisella novicida
atggattattacttaactggagtgtttac

SEQ ID NO: 26 - DNA, 45 bp, Francisella novicida
aatgttcaatggattattacttaattggagtgtctacgtcgatgg

SEQ ID NO: 27 - DNA, 28 bp, Francisella novicida
gccacaaatactacaaaaaataacttaa

SEQ ID NO: 28 - DNA, 44 bp, Francisella novicida
attttttggctccaaatactacaaaaaataacttaaactttgaa

SEQ ID NO: 29 - DNA, 32 bp, Francisella novicida
attgtcaaaacataagcagctgcttcaaatat

SEQ ID NO: 30 - DNA, 48 bp, Francisella novicida
ggtcttttactgttattacataagcagccgcttcaaatatcttagcaa

SEQ ID NO: 31 - protein, 10 aa, Artificial Sequence
  An isolated polypeptide or fragment thereof  having a nuclease activity.
YLFQIYNKDF

SEQ ID NO: 32 - protein, 1184 aa, Methanomethylophilus alvus
MDAKEFTGQYPLSKTLRFELRPIGRTWDNLEASGYLAEDRHRAECYPRAKELLDDNHRAFLNRVLPQIQDADGYKGLFAKPALDEAMKIAKENGNESDIEVLEAFNGFSVYFTGYHESRENIYSDEDMVSVAYRITEDNFPRFVSNALIFDKLNESHPDIISEVSGNLGVDDIGKYFDVSNYNNFLSQAGIDDYNHIIGGHTTEDGLIQAFNVVLNLRHQKDPGFEKIQFKQLYKQILSVRTSKSYIPKQFDNSKEMVDCICDYVSKIEKSETVERALKLVRNISSFDLRGIFVNKKNLRILSNKLIGDWDAIETALMHSSSSENDKKSVYDSAEAFTLDDIFSSVKKFSDASAEDIGNRAEDICRVISETAPFINDLRAVDLDSLNDDGYEAAVSKIRESLEPYMDLFHELEIFSVGDEFPKCAAFYSELEEVSEQLIEIIPLFNKARSFCTRKRYSTDKIKVNLKFPTLADGWDLNKERDNKAAILRKDGKYYLAILDMKKDLSSIRTSDEDESSFEKMEYKLLPSPVKMLPKIFVKSKAAKEKYGLTDRMLECYDKGMHKSGSAFDLGFCHELIDYYKRCIAEYPGWDVFDFKFRETSDYGSMKEFNEDVAGAGYYMSLRKIPCSEVYRLLDEKSIYLFQIYNKDYSENAHGNKNMHTMYWEGLFSPQNLESPVFKLSGGAELFFRKSSIPNDAKTVHPKGSVLVPRNDVNGRRIPDSIYRELTRYFNRGDCRISDEAKSYLDKVKTKKADHDIVKDRRFTVDKMMFHVPIAMNFKAISKPNLNKKVIDGIIDDQDLKIIGIDRGERNLIYVTMVDRKGNILYQDSLNILNGYDYRKALDVREYDNKEARRNWTKVEGIRKMKEGYLSLAVSKLADMIIENNAIIVMEDLNHGFKAGRSKIEKQVYQKFESMLINKLGYMVLKDKSIDQSGGALHGYQLANHVTTLASVGKQCGVIFYIPAAFTSKIDPTTGFADLFALSNVKNVASMREFFSKMKSVIYDKAEGKFAFTFDYLDYNVKSECGRTLWTVYTVGERFTYSRVNREYVRKVPTDIIYDALQKAGISVEGDLRDRIAESDGDTLKSIFYAFKYALDMRVENREEDYIQSPVKNASGEFFCSKNAGKSLPQDSDANGAYNIALKGILQLRMLSEQYDPNAESIRLPLITNKAWLTFMQSGMKTWK

SEQ ID NO: 33 - protein, 1265 aa, Acidaminococcus sp. BV3L6 8
MTQFEGFTNLYQVSKTLRFELIPQGKTLKHIQEQGFIEEDKARNDHYKELKPIIDRIYKTYADQCLQLVGRTDNLTDAINKRHAEIYKGLFKAELFNGKVLKQLGTVTTTEHENALLRSFDKFTTYFSGFYENRKNVFSAEDISTAIPHRIVQDNFPKFKENCHIFTRLITAVPSLREHFENVKKAIGIFVSTSIEEVFSFPFYNQLLTQTQIDLYNQLLGGISREAGTEKIKGLNEVLNLAIQKNDETAHIIASLPHRFIPLFKQILSDRNTLSFILEEFKSDEEVIQSFCKYKTLLRNENVLETAEALFNELNSIDLTHIFISHKKLETISSALCDHWDTLRNALYERRISELTGKITKSAKEKVQRSLKHEDINLQEIISAAGKELSEAFKQKTSEILSHAHAALDQPLPTTLKKQEEKEILKSQLDSLLGLYHLLDWFAVDESNEVDPEFSARLTGIKLEMEPSLSFYNKARNYATKKPYSVEKFKLNFQMPTLASGWDVNKEKNNGAILFVKNGLYYLGIMPKQKGRYKALSFEPTEKTSEGFDKMYYDYFPDAAKMIPKCSTQLKAVTAHFQTHTTPILLSNNFIEPLEITKEIYDLNNPEKEPKKFQTAYAKKTGDQKGYREALCKWIDFTRDFLSKYTKTTSIDLSSLRPSSQYKDLGEYYAELNPLLYHISFQRIAEKEIMDAVETGKLYLFQIYNKDFAKGHHGKPNLHTLYWTGLFSPENLAKTSIKLNGQAELFYRPKSRMKRMAHRLGEKMLNKKLKDQKTPIPDTLYQELYDYVNHRLSHDLSDEARALLPNVITKEVSHEIIKDRRFTSDKFFFHVPITLNYQAANSPSKFNQRVNAYLKEHPETPIIGIDRGERNLIYITVIDSTGKILEQRSLNTIQQFDYQKKLDNREKERVAARQAWSVVGTIKDLKQGYLSQVIHEIVDLMIHYQAVVVLENLNFGFKSKRTGIAEKAVYQQFEKMLIDKLNCLVLKDYPAEKVGGVLNPYQLTDQFTSFAKMGTQSGFLFYVPAPYTSKIDPLTGFVDPFVWKTIKNHESRKHFLEGFDFLHYDVKTGDFILHFKMNRNLSFQRGLPGFMPAWDIVFEKNETQFDAKGTPFIAGKRIVPVIENHRFTGRYRDLYPANELIALLEEKGIVFRDGSNILPKLLENDDSHAIDTMVALIRSVLQMRNSNAATGEDYINSPVRDLNGVCFDSRFQNPEWPMDADANGAYHIALKGQLLLNHLKESKDLKLQNGISNQDWLAYIQELRN

SEQ ID NO: 34 - protein, 1187 aa, Lachnospiraceae
MSKLEKFTNCYSLSKTLRFKAIPVGKTQENIDNKRLLVEDEKRAEDYKGVKKLLDRYYLSFINDVLHSIGNEGYKSLFKKDIIETILPEFLDDKDEIALVNSFNGFTTAFTGFFDNRENMFSEEAKSTSIAFRCINENLTRYISNMDIFEKVDAIFDKHEVQEIKEKILNSDYDVEDFFEGEFFNFVLTQEGIDVYNAIIGGFVTESGEKIKGLNEYINLYNQKTKQKLPKFKPLYKQVLSDRESLSFYGEGYTSDEEVLEVFRNTLNKNSEIFSSIKKLEKLFKNFDEYSSAGIFVKNGPAISTISKDIFGEWNVIRDKWNAEYDDIHLKKKAVVTEKYEDDRRKSFKKIGSFSLEQLQEYADADLSVVEKLKEIIIQKVDEIYKVYGSSEKLFDADFVLEKSLKKNDAVVAIMKDLLDSVKSFENYIKAFFGEGKETNRDESFYGDFVLAYDILLKVDHIYDAIRNYVTQKPYSKDKFKLYFQNPQFMGGWDKDKETDYRATILRYGSKYYLAIMDKKYAKCLQKIDKDDVNGNYEKINYKLLPGPNKMLPKVFFSKKWMAYYNPSEDIQKIYKNGTFKKGDMFNLNDCHKLIDFFKDSISRYPKWSNAYDFNFSETEKYKDIAGFYREVEEQGYKVSFESASKKEVDKLVEEGKLYMFQIYNKDFSDKSHGTPNLHTMYFKLLFDENNHGQIRLSGGAELFMRRASLKKEELVVHPANSPIANKNPDNPKKTTTLSYDVYKDKRFSEDQYELHIPIAINKCPKNIFKINTEVRVLLKHDDNPYVIGIDRGERNLLYIVVVDGKGNIVEQYSLNEIINNFNGIRIKTDYHSLLDKKEKERFEARQNWTSIENIKELKAGYISQVVHKICELVEKYDAVIALEDLNSGFKNSRVKVEKQVYQKFEKMLIDKLNYMVDKKSNPCATGGALKGYQITNKFESFKSMSTQNGFIFYIPAWLTSKIDPSTGFVNLLKTKYTSIADSKKFISSFDRIMYVPEEDLFEFALDYKNFSRTDADYIKKWKLYSYGNRIRIFRNPKKNNVFDWEEVCLTSAYKELFNKYGINYQQGDIRALLCEQSDKAFYSSFMALMSLMLQMRNSITGRTDVDFLISPVKNSDGIFYDSRNYEAQENAILPKNADANGAYNIARKVLWAIGQFKKAEDEKLDKVKIAISNKEWLEYAQTSVKH

SEQ ID NO: 35 - protein, 1255 aa, Francisella tularensis U112 1
MSIYQEFVNKYSLSKTLRFELIPQGKTLENIKARGLILDDEKRAKDYKKAKQIIDKYHQFFIEEILSSVDSEKFKNLFNQNLIDAKKGQESDLILWLKQSKDNGIELFKANSDITDIDEALEIIKSFKGWTTYFKGFHENRKNVYSSNDIPTSIIYRIVDDNLPKFLENKAKYESLKDKAPEAINYEQIKKDLAEELTFDIDYKTSEVNQRVFSLDEVFEIANFNNYLNQSGITKFNTIIGGKFVNGENTKRKGINEYINLYSQQINDKTLKKYKMSVLFKQILSDTESKSFVIDKLEDDSDVVTTMQSFYEQIAAFKTVEEKSIKETLSLLFDDLKAQKLDLSKIYFKNDKSLTDLSQQVFDDYSVIGTAVLEYITQQIAPKNLDNPSKKEQELIAKKTEKAKYLSLETIKLALEEFNKHRDIDKQCRFEEILANFAAIPMIFDEIAQNKDNLAQISIKYQNQGKKDLLQASAEDDVKAIKDLLDQTNNLLHKLKIFHISQSEDKANILDKDEHFYLVFEECYFELANIVPLYNKIRNYITQKPYSDEKFKLNFENSTLANGWDKNKEPDNTAILFIKDDKYYLGVMNKKNNKIFDDKAIKENKGEGYKKIVYKLLPGANKMLPKVFFSAKSIKFYNPSEDILRIRNHSTHTKNGSPQKGYEKFEFNIEDCRKFIDFYKQSISKHPEWKDFGFRFSDTQRYNSIDEFYREVENQGYKLTFENISESYIDSVVNQGKLYLFQIYNKDFSAYSKGRPNLHTLYWKALFDERNLQDVVYKLNGEAELFYRKQSIPKKITHPAKEAIANKNKDNPKKESVFEYDLIKDKRFTEDKFFFHCPITINFKSSGANKFNDEINLLLKEKANDVHILSIDRGERHLAYYTLVDGKGNIIKQDTFNIIGNDRMKTNYHDKLAAIEKDRDSARKDWKKINNIKEMKEGYLSQVVHEIAKLVIEYNAIVVFEDLNFGFKRGRFKVEKQVYQKLEKMLIEKLNYLVFKDNEFDKTGGVLRAYQLTAPFETFKKMGKQTGIIYYVPAGFTSKICPVTGFVNQLYPKYESVSKSQEFFSKFDKICYNLDKGYFEFSFDYKNFGDKAAKGKWTIASFGSRLINFRNSDKNHNWDTREVYPTKELEKLLKDYSIEYGHGECIKAAICGESDKKFFAKLTSVLNTILQMRNSKTGTELDYLISPVADVNGNFFDSRQAPKNMPQDADANGAYHIGLKGLMLLGRIKNNQEGKKLNLVIKNEEYFEFVQNRNN

SEQ ID NO: 36 - protein, 1196 aa, Candidatus Methanoplasma termitum 10
MNNYDEFTKLYPIQKTIRFELKPQGRTMEHLETFNFFEEDRDRAEKYKILKEAIDEYHKKFIDEHLTNMKDDRFKDLFSKKLFSELLKEEIYKKGNHQEIDALKSFDKFSGYFIGLHENRKNMYSDGDEITAISNRIVNENFPKFLDNLQKYQEARKKYPEWIIKAESALVAHNIKMDEVFSLEYFNKVLNQEGIQRYNLALGGYVTKSGEKMMGLNDALNLAHQSEKSSKGRIHMTPLFKQILSEKESFSYIPDVFTEDSQLLPSIGGFFAQIENDKDGNIFDRALELISSYAEYDTERIYIRQADINRVSNVIFGEWGTLGGLMREYKADSINDINLERTCKKVDKWLDSKEFALSDVLEAIKRTGNNDAFNEYISKMRTAREKIDAARKEMKFISEKISGDEESIHIIKTLLDSVQQFLHFFNLFKARQDIPLDGAFYAEFDEVHSKLFAIVPLYNKVRNYLTKNNLNTKKIKLNFKNPTLANGWDQNKVYDYASLIFLRDGNYYLGIINPKRKKNIKFEQGSGNGPFYRKMVYKQIPGPNKNLPRVFLTSTKGKKEYKPSKEIIEGYEADKHIRGDKFDLDFCHKLIDFFKESIEKHKDWSKFNFYFSPTESYGDISEFYLDVEKQGYRMHFENISAETIDEYVEKGDLFLFQIYNKDFVKAATGKKDMHTIYWNAAFSPENLQDVVVKLNGEAELFYRDKSDIKEIVHREGEILVNRTYNGRTPVPDKIHKKLTDYHNGRTKDLGEAKEYLDKVRYFKAHYDITKDRRYLNDKIYFHVPLTLNFKANGKKNLNKMVIEKFLSDEKAHIIGIDRGERNLLYYSIIDRSGKIIDQQSLNVIDGFDYREKLNQREIEMKDARQSWNAIGKIKDLKEGYLSKAVHEITKMAIQYNAIVVMEELNYGFKRGRFKVEKQIYQKFENMLIDKMNYLVFKDAPDESPGGVLNAYQLTNPLESFAKLGKQTGILFYVPAAYTSKIDPTTGFVNLFNTSSKTNAQERKEFLQKFESISYSAKDGGIFAFAFDYRKFGTSKTDHKNVWTAYTNGERMRYIKEKKRNELFDPSKEIKEALTSSGIKYDGGQNILPDILRSNNNGLIYTMYSSFIAAIQMRVYDGKEDYIISPIKNSKGEFFRTDPKRRELPIDADANGAYNIALRGELTMRAIAEKFDPDSEKMAKLELKHKDWFEFMQTRGD